European Patent Specification EP 3 299 383 B1, published December 3, 2025. Title: Specific modification of an antibody with an IgG binding peptide. Applicant: Kagoshima University. The sequence listing filed with the application follows.

SEQUENCE LISTING (37 sequences)

SEQ ID NO: 1 - protein, 13 aa, Artificial
  IgG-binding peptide
  misc_feature (6)..(6): Xaa is lysine, cystein, aspartic acid, glutamic acid, 2-amino suberic acid, or diaminopropionic acid
DCAYHXGELVWCT

SEQ ID NO: 2 - protein, 17 aa, Artificial
  IgG-binding peptide
  misc_feature (8)..(8): Xaa is lysine, cystein, aspartic acid, glutamic acid, 2-amino suberic acid, or diaminopropionic acid
GPDCAYHXGELVWCTFH

SEQ ID NO: 3 - protein, 13 aa, Artificial
  IgG-binding peptide
  misc_feature (6)..(6): Xaa is lysine, cystein, aspartic acid, glutamic acid, 2-amino suberic acid, or diaminopropionic acid
RCAYHXGELVWCS

SEQ ID NO: 4 - protein, 17 aa, Artificial
  IgG-binding peptide
  misc_feature (8)..(8): Xaa is lysine, cystein, aspartic acid, glutamic acid, 2-amino suberic acid, or diaminopropionic acid
GPRCAYHXGELVWCSFH

SEQ ID NO: 5 - protein, 17 aa, Artificial
  IgG-binding peptide
  misc_feature (8)..(8): Xaa is lysine, cystein, aspartic acid, glutamic acid, 2-amino suberic acid, or diaminopropionic acid
SPDCAYHXGELVWCTFH

SEQ ID NO: 6 - protein, 17 aa, Artificial
  IgG-binding peptide
  misc_feature (8)..(8): Xaa is lysine, cystein, aspartic acid, glutamic acid, 2-amino suberic acid, or diaminopropionic acid
GDDCAYHXGELVWCTFH

SEQ ID NO: 7 - protein, 17 aa, Artificial
  IgG-binding peptide
  misc_feature (8)..(8): Xaa is lysine, cystein, aspartic acid, glutamic acid, 2-amino suberic acid, or diaminopropionic acid
GPSCAYHXGELVWCTFH

SEQ ID NO: 8 - protein, 17 aa, Artificial
  IgG-binding peptide
  misc_feature (8)..(8): Xaa is lysine, cystein, aspartic acid, glutamic acid, 2-amino suberic acid, or diaminopropionic acid
GPDCAYHXGELVWCSFH

SEQ ID NO: 9 - protein, 17 aa, Artificial
  IgG-binding peptide
  misc_feature (8)..(8): Xaa is lysine, cystein, aspartic acid, glutamic acid, 2-amino suberic acid, or diaminopropionic acid
GPDCAYHXGELVWCTHH

SEQ ID NO: 10 - protein, 17 aa, Artificial
  IgG-binding peptide
  misc_feature (8)..(8): Xaa is lysine, cystein, aspartic acid, glutamic acid, 2-amino suberic acid, or diaminopropionic acid
GPDCAYHXGELVWCTFY

SEQ ID NO: 11 - protein, 17 aa, Artificial
  IgG-binding peptide
  misc_feature (8)..(8): Xaa is lysine, cystein, aspartic acid, glutamic acid, 2-amino suberic acid, or diaminopropionic acid
SPDCAYHXGELVWCTFY

SEQ ID NO: 12 - protein, 17 aa, Artificial
  IgG-binding peptide
  misc_feature (8)..(8): Xaa is lysine, cystein, aspartic acid, glutamic acid, 2-amino suberic acid, or diaminopropionic acid
SDDCAYHXGELVWCTFY

SEQ ID NO: 13 - protein, 17 aa, Artificial
  IgG-binding peptide
  misc_feature (8)..(8): Xaa is lysine, cystein, aspartic acid, glutamic acid, 2-amino suberic acid, or diaminopropionic acid
RGNCAYHXGQLVWCTYH

SEQ ID NO: 14 - protein, 13 aa, Artificial
  IgG-binding peptide
  misc_feature (6)..(6): Xaa is lysine, cystein, aspartic acid, glutamic acid, 2-amino suberic acid, or diaminopropionic acid
DCTYHXGNLVWCT

SEQ ID NO: 15 - protein, 13 aa, Artificial
  IgG-binding peptide
  misc_feature (6)..(6): Xaa is lysine, cystein, aspartic acid, glutamic acid, 2-amino suberic acid, or diaminopropionic acid
DCAYHXGNLVWCT

SEQ ID NO: 16 - protein, 13 aa, Artificial
  IgG-binding peptide
  misc_feature (6)..(6): Xaa is lysine, cystein, aspartic acid, glutamic acid, 2-amino suberic acid, or diaminopropionic acid
DCTYHXGELVWCT

SEQ ID NO: 17 - protein, 13 aa, Artificial
  IgG-binding peptide
  misc_feature (6)..(6): Xaa is lysine, cystein, aspartic acid, glutamic acid, 2-amino suberic acid, or diaminopropionic acid
DCAWHXGELVWCT

SEQ ID NO: 18 - protein, 13 aa, Artificial
  IgG-binding peptide
  misc_feature (6)..(6): Xaa is lysine, cystein, aspartic acid, glutamic acid, 2-amino suberic acid, or diaminopropionic acid
DCTYTXGNLVWCT

SEQ ID NO: 19 - protein, 13 aa, Artificial
  IgG-binding peptide
  misc_feature (6)..(6): Xaa is lysine, cystein, aspartic acid, glutamic acid, 2-amino suberic acid, or diaminopropionic acid
DCAYTXGNLVWCT

SEQ ID NO: 20 - protein, 13 aa, Artificial
  IgG-binding peptide
  misc_feature (6)..(6): Xaa is lysine, cystein, aspartic acid, glutamic acid, 2-amino suberic acid, or diaminopropionic acid
DCSYTXGNLVWCT

SEQ ID NO: 21 - protein, 13 aa, Artificial
  IgG-binding peptide
  misc_feature (6)..(6): Xaa is lysine, cystein, aspartic acid, glutamic acid, 2-amino suberic acid, or diaminopropionic acid
DCTWTXGNLVWCT

SEQ ID NO: 22 - protein, 13 aa, Artificial
  IgG-binding peptide
  misc_feature (6)..(6): Xaa is lysine, cystein, aspartic acid, glutamic acid, 2-amino suberic acid, or diaminopropionic acid
DCTYHXGNLVWCT

SEQ ID NO: 23 - protein, 13 aa, Artificial
  IgG-binding peptide
  misc_feature (6)..(6): Xaa is lysine, cystein, aspartic acid, glutamic acid, 2-amino suberic acid, or diaminopropionic acid
DCTYRXGNLVWCT

SEQ ID NO: 24 - protein, 13 aa, Artificial
  IgG-binding peptide
  misc_feature (6)..(6): Xaa is lysine, cystein, aspartic acid, glutamic acid, 2-amino suberic acid, or diaminopropionic acid
DCTYSXGNLVWCT

SEQ ID NO: 25 - protein, 13 aa, Artificial
  IgG-binding peptide
  misc_feature (6)..(6): Xaa is lysine, cystein, aspartic acid, glutamic acid, 2-amino suberic acid, or diaminopropionic acid
DCTYTXGNLVWCT

SEQ ID NO: 26 - protein, 13 aa, Artificial
  IgG-binding peptide
  misc_feature (6)..(6): Xaa is lysine, cystein, aspartic acid, glutamic acid, 2-amino suberic acid, or diaminopropionic acid
DCTYTXGELVWCT

SEQ ID NO: 27 - protein, 13 aa, Artificial
  IgG-binding peptide
  misc_feature (6)..(6): Xaa is lysine, cystein, aspartic acid, glutamic acid, 2-amino suberic acid, or diaminopropionic acid
DCTYTXGRLVWCT

SEQ ID NO: 28 - protein, 13 aa, Artificial
  IgG-binding peptide
  misc_feature (6)..(6): Xaa is lysine, cystein, aspartic acid, glutamic acid, 2-amino suberic acid, or diaminopropionic acid
DCTYTXGDLVWCT

SEQ ID NO: 29 - protein, 13 aa, Artificial
  IgG-binding peptide
  misc_feature (6)..(6): Xaa is lysine, cystein, aspartic acid, glutamic acid, 2-amino suberic acid, or diaminopropionic acid
DCTYTXGNLIWCT

SEQ ID NO: 30 - protein, 110 aa, Homo Sapiens
APELLGGPSVFLFPPKPKDTLMISRTPEVTCVVVDVSHEDPEVKFNWYVDGVEVHNAKTKPREEQYNSTYRVVSVLTVLHQDWLNGKEYKCKVSNKALPAPIEKTISKAK

SEQ ID NO: 31 - protein, 17 aa, Artificial
  IgG-binding peptide
  misc_feature (2)..(2): Xaa is homoserine
  misc_feature (16)..(16): Xaa is homoserine
GXDCAYHRGELVWCTXH

SEQ ID NO: 32 - protein, 17 aa, Artificial
  IgG-binding peptide
  misc_feature (8)..(8): Xaa is lysine, cystein, aspartic acid, glutamic acid, 2-amino suberic acid, or diaminopropionic acid
GPDCAYHXGELVWCTFH

SEQ ID NO: 33 - protein, 13 aa, Artificial
  IgG-binding peptide
DCAYHRGELVWCT

SEQ ID NO: 34 - protein, 13 aa, Artificial
  IgG-binding peptide
DCAYHKGELVWCT

SEQ ID NO: 35 - protein, 17 aa, Artificial
  IgG-binding peptide
  misc_feature (8)..(8): Xaa is lysine, cystein, aspartic acid, glutamic acid, 2-amino suberic acid, or diaminopropionic acid
RGNCAYHXGQLVWCTYH

SEQ ID NO: 36 - protein, 17 aa, Artificial
  IgG-binding peptide
  misc_feature (2)..(2): Xaa is homoserine
  misc_feature (8)..(8): Xaa is lysine, cystein, aspartic acid, glutamic acid, 2-amino suberic acid, or diaminopropionic acid
  misc_feature (16)..(16): Xaa is homoserine
GXDCAYHXGELVWCTXH

SEQ ID NO: 37 - protein, 19 aa, Artificial
  IgG-binding peptide
  misc_feature (10)..(10): Xaa is lysine, cystein, aspartic acid, glutamic acid, 2-amino suberic acid, or diaminopropionic acid
RRGPDCAYHXGELVWCTFH